European Patent Specification EP 3 800 259 B1, published March 20, 2024. Title: AXMI477, AXMI482, AXMI486 AND AXMI525 TOXIN GENES AND METHODS FOR THEIR USE. Applicant: BASF Agricultural Solutions Seed US LLC. The sequence listing filed with the application follows.

SEQUENCE LISTING (27 sequences)

SEQ ID NO: 1 - DNA, 3695 bp, Bacillus thuringiensis
atgaatcgaaataatcaaggtgaatatgaaattattgacgcttccacttgtggttgttcgtcagatgatgttgttcaatatcctttggcaagagatccgaatgctgcattccaaaatatgaattataaagattatttgaaaatgtctgacggagactacgtcgattcttatataaacccaggcttatctattggtcgtagagatgtgaccctaactggagttggtattgttgcgctaatagtagggactttaggtggtccagttgggggtatagtaactggcttgatttcctctcttttaggattattgtggccaagtaatgataatgatgtatgggaagcttttatggcacaaatagaagagctaattgaacaaaggatagcagatcaagtagtaaggaatgcactcgataacttaactggattgcgcgattattataatcaatacctattagcattggaggagtggcaggaaaggccgaacgctgtaagatctaccttagtttttaatagatttgaaaccctgcattctcactttgtaactagtatgccaagctttggtagtggccctggaagtgaaaggtatgcggtacaattgctgacagtttatgcacaagcggcaaatctgcatttgttattattaagagatgctgacatttatggggcaaggtggggacttcgtgaatctcagattgatttatattttaatgagctacaaaatcgtactcgagattataccaatcattgtgtaactgcgtacaataatgggttagaggagatacgaggaacaagccctgcaagttggttgaggtaccatcaattccgtagagagacaacactaatagcattggatttagtggcgatattcccatattacaacgtacgagaatatccaattggggtaaatcctcagcttacacgtgatgtatatacagatccaataggggttactttcagaagagaagattgggaaacaggagtagaatgcagaccatgggtaaatactccttacatgagcttttcggatcttgaaaatgcaataattcgtccaccacatctatttgaaacattacgtaatttaacaattcatacaggtcgatataacctagtaggaggggcgagatttattgaaggatgggtcggacattctgtaacaaatactcgcttgggtaattcaacagtatttacaagtaattatggttctttgccacctcgttttcaagtttttaattttactaattttgatgtttaccaaattaatacgagagcagattctacaggtacctttagaatccctggatttgcagttacaagggcccaattcattccgggtgggacttattcagtagctcaccgagatccaggggcatgtcaacaagattatgattcaattgaagagttaccaagtctagacccggatgaacctattaatagaagttatagtcatagattatcgcatgttaccctttataaatatactctctcagatacagattatggagttatcaattatacagattatggaagtatgcctgcatatgtctggacacatcgcgatgtggaccttactaacacgattactgcagatagaattacacaactcccattagtaaaggcatctacactacctgcgggtactactgtggtaaaaggcccaggatttacaggaggagatatactccgaagaacaactaatggaacatttgggacattacatgtaagggttaattcaccattaacacaacaatatcgcctaagagttcgttttgcctcaacaggaaatttcagtataagggtactccgtggagggacttctatcggtgatgctagatttgggagcacaatgaacagaggacaggaactaacttacgaatcctttgtcacaagagagtttactactactggtccgttcaatccgccttttacatttacacaaactcaagaaattctaacagtgaatgcagaaggtgttagcaccggtggtgaatattatatagatagtattgagattgttcctgtaaatccgacgcgagaggcggaagaggatctagaagcagcgaagaaagcggtggcgagcttgtttacacgtacaagggacggattacaagtaaatgtgacagattatcaagtcgatcaagcggcaaatttagtgtcatgcttatcagatgaacaatatgggcatgacaaaaagatgttattggaagcggtaagagcggcaaaacgcctcagccgagaacgcaacttacttcaggatccagattttaatacaatcaatagtacagaagaaaatggatggaaagcaagtaacggcgttactattagcgagggcggtccattctataaaggccgtgcgcttcagctagcaagcgcaagagaaaattacccaacatacatttatcaaaaagtaaatgcatcagagttaaagccgtatacacgttatagactggatgggttcgtgaagagtagtcaagatttagaaattgatctcattcaccatcataaagtccatctcgtgaaaaatgtaccagataatttagtatccgatacttactcggatggttcttgcagtggaatgaatcgatgtgaggaacaacagatggtaaatgcgcaactggaaacagaacatcatcatccgatggattgctgtgaagcggctcaaacacatgagttttcttcctatattaatacaggcgatctaaattcaagtgtagatcaaggcatttgggttgtattgaaagttcgaacaaccgatggttatgcgacgctaggaaatcttgaattggtagaggtcggaccgttatcgggtgaatctctagaacgtgaacaaagggataatgcgaaatggagtgcagagctaggaagaaagcgtgcagaaacagatcgcgtgtatcaagatgccaaacaatccatcaatcatttatttgtggattatcaagatcaacaattaaatccagaaatagggatggcagatattattgacgctcaaaatcttgtcgcatcaatttcagatgtgtatagcgatgcagtactgcaaatccctggaattaactatgagatttacacagagctatccaatcgcttacaacaagcatcgtatctgtatacgtctcgaaatgcggtgcaaaatggggactttaacagcggtctagatagttggaatgcaacagggggggctacggtacaacaggatggcaatacgcatttcttagttctttctcattgggatgcacaagtttctcaacaatttagagtgcagccgaattgtaaatatgtattacgtgtaacagcagagaaagtaggcggcggagacggatacgtgacaatccgggatggtgctcatcatacagaaaagcttacatttaatgcatgtgattatgatataaatggcacgtacgtgactgataatacgtatctaacaaaagaagtggtattctattcacatacagaacacatgtgggtagaggtaagtgaaacagaaggtgcatttcatatagatagtattgaattcgttgaaacagaaaagtaacgggatgatgttccgaacatataaggtataaggaacgatacgccgtataaaagattctcaaacagaatgtgaaataaatgaggacccctccgggtagtcgtacatggaaagtacacgactacccggagggtattttttatataaaaaatgtggtttttcactacggtcta

SEQ ID NO: 2 - DNA, 1008 bp, Bacillus thuringiensis
atgaataaaaaagtaacaaaaacagtattaagcgtggtaatgggtataagtgttttagcatctcctttagctgtagccgcaaaaacagagaataataaagaacaacaagtaattacacagtttaatcagagagaaaataagttccctgatgtaggacaggggattcaatggttatctcaattttatggaaaatctttaaagaataatggtgaaggatactccttaggtaatgatgtaatgagctattttttagaagtaaagaattcttatggtcaattggcaatagaacctcaagtaataagcactacacctctttgggctggccaaagcgacttggaaaatgcaactgatcatgaacaaactttaaattccacagaatttaaaaaaacgtattctaacacaaccaccacctctacagaaaatggatttatgataggtcaggaaaccgaagggaaagttggtataccctttgtcgcagaaggaaaagtcaccataaaaactgaatataactttaatcatactaatgggtatgaaacatctgaaagtgtagagtatattgctccttctcaatctattaaggtaccaccgcatactattgcccgagtgacagcattattagatgtgaaaaaaattaaaggaaagatgcatctatattcagaaattgggcttaataaagattatggttacgatatggtgccacttgtttataaatatggaggaccatttaagtatgtaaccttaggcacattatatgacgagggctataagcaggcacaattagattattccaatatgggaaatgttataccggaagaaattgagactgtttcgaaaagtaacaatcccaaccatttattagcaagtggattaggaatctttgaatcagaatacggaagtgtatttaatgttaaagttgaatacattaatattaaaactaaaaagattgaaaaaacagagaatcttactattgaacctacaatagtccctgttgaaaagacgaatacaaaa

SEQ ID NO: 3 - DNA, 1023 bp, Bacillus thuringiensis
gtgagggagaaggatttgaataaaaaagtaacaaaggcagtattaagcatgatagtgggtataagtgttttagcatctcctttagctgtagccgcaaaaacagagaataataaagaacaacaagtaattacacattttaatcagagagaaaataagttccctgatgtaggacaggggattcaatggttatctcaattttatggaaagtctttaaagaataatggtgaaggatactccttaggtcaggatgtaatgagatattttttagaagtaaagaattcttacggtcaattggcaatggaacctcaagtaataagcactacacctctttgggccggccaaagtgacttggaaaatgcaactgatcatgaacaaactttaaattccacagaatttaaaaaaacgtattctaacacaacaaccacctctacagaaaatggatttatgataggtcaagagactgaagggaaagttggtattccctttgtcgcagaaggaaaagtcaccataaaaactgaatataactttaatcatactaatgggtatgaaacatctgaaagtgtagagtatattgctccttctcaatctattaaggtaccaccgcatactattgcccgagtgacagcattattagatgtgaaaaaaatcaaagggaaaatgcatctatattcagaaattgggcttaataaagattatggttacgatatggtgccacttgtttataaatatggaggtccatttaagtatgtaaccttaggcacattatatgacgagggctataagcaggcacaattagattatttcaatatgggaaatgttataccggaagaaattgagactgtttcaaaaagtaacaatcccaaccatttattagcaagtggagtaggaatctttgaatcagaatacggaagtgtatttaatgttaaagttgaatacattaatattaatacgaaaaagattgaaaaaacagagaatcttactattgaacctacaatagtccctgttaaacagacgaatacaaaa

SEQ ID NO: 4 - DNA, 1029 bp, Bacillus thuringiensis
gtgagggagaaagatatggataaaaaaataacaaaagcagcgttaagcatgataatgggtataagtgttttatcatctcctttagctgtagccgcaaaaacagagaataataaagaacaacacgtaattacacagtttaatcagagagaaaataagttccctgatgtaggacaggggattcaatggttatctcaattttatggaaaatctttaaagaataatggggaaggatactccttaggtcaggatgtaatgagctattttctagaagtaaaaaattcttatggtcaattggcaatggaacctcaagtaataagcactacacctctttgggctggccaaagtgacttggaaaatgcaactgatcatgaacaaactttaaattccacagaatttaaaaaaacgtattctaacacaacaaccacctctacagaaaatggatttatgataggtcaagagactgaagggaaagttggtattccctttgtcgcagaaggaaaagtcaccataaaaactgaatataactttaatcatactaatgggtatgaaacatctgaaagtgtagagtatattgctccttctcaatctattaaggtaccaccgcatactattgcccgagtgacagcattattagatgtgaaaaaaatcaaagggaaaatgcatctatattcagaaattgggcttaataaagattatggttacgatatggtgccacttgtttataaatatggaggtccatttaagtatgtaaccttaggcacattatatgacgagggctataagcaggcacaattagattatttcaatatgggaaatgttataccggaagaaattgagactgtttcaaaaagtaacaatcccaaccatttattagcaagtggagtaggaatctttgaatcagaatacggaagtgtatttaatgttaaagttgaatacattaatattaatacgaaaaagattgaaaaaacagagaatcttactattgaacctacaatagtccctgttaaacagacgaatacgaatacaaaa

SEQ ID NO: 5 - protein, 1174 aa, Bacillus thuringiensis
MNRNNQGEYEIIDASTCGCSSDDVVQYPLARDPNAAFQNMNYKDYLKMSDGDYVDSYINPGLSIGRRDVTLTGVGIVALIVGTLGGPVGGIVTGLISSLLGLLWPSNDNDVWEAFMAQIEELIEQRIADQVVRNALDNLTGLRDYYNQYLLALEEWQERPNAVRSTLVFNRFETLHSHFVTSMPSFGSGPGSERYAVQLLTVYAQAANLHLLLLRDADIYGARWGLRESQIDLYFNELQNRTRDYTNHCVTAYNNGLEEIRGTSPASWLRYHQFRRETTLIALDLVAIFPYYNVREYPIGVNPQLTRDVYTDPIGVTFRREDWETGVECRPWVNTPYMSFSDLENAIIRPPHLFETLRNLTIHTGRYNLVGGARFIEGWVGHSVTNTRLGNSTVFTSNYGSLPPRFQVFNFTNFDVYQINTRADSTGTFRIPGFAVTRAQFIPGGTYSVAHRDPGACQQDYDSIEELPSLDPDEPINRSYSHRLSHVTLYKYTLSDTDYGVINYTDYGSMPAYVWTHRDVDLTNTITADRITQLPLVKASTLPAGTTVVKGPGFTGGDILRRTTNGTFGTLHVRVNSPLTQQYRLRVRFASTGNFSIRVLRGGTSIGDARFGSTMNRGQELTYESFVTREFTTTGPFNPPFTFTQTQEILTVNAEGVSTGGEYYIDSIEIVPVNPTREAEEDLEAAKKAVASLFTRTRDGLQVNVTDYQVDQAANLVSCLSDEQYGHDKKMLLEAVRAAKRLSRERNLLQDPDFNTINSTEENGWKASNGVTISEGGPFYKGRALQLASARENYPTYIYQKVNASELKPYTRYRLDGFVKSSQDLEIDLIHHHKVHLVKNVPDNLVSDTYSDGSCSGMNRCEEQQMVNAQLETEHHHPMDCCEAAQTHEFSSYINTGDLNSSVDQGIWVVLKVRTTDGYATLGNLELVEVGPLSGESLEREQRDNAKWSAELGRKRAETDRVYQDAKQSINHLFVDYQDQQLNPEIGMADIIDAQNLVASISDVYSDAVLQIPGINYEIYTELSNRLQQASYLYTSRNAVQNGDFNSGLDSWNATGGATVQQDGNTHFLVLSHWDAQVSQQFRVQPNCKYVLRVTAEKVGGGDGYVTIRDGAHHTEKLTFNACDYDINGTYVTDNTYLTKEVVFYSHTEHMWVEVSETEGAFHIDSIEFVETEK

SEQ ID NO: 6 - protein, 1135 aa, Bacillus thuringiensis
MNYKDYLKMSDGDYVDSYINPGLSIGRRDVTLTGVGIVALIVGTLGGPVGGIVTGLISSLLGLLWPSNDNDVWEAFMAQIEELIEQRIADQVVRNALDNLTGLRDYYNQYLLALEEWQERPNAVRSTLVFNRFETLHSHFVTSMPSFGSGPGSERYAVQLLTVYAQAANLHLLLLRDADIYGARWGLRESQIDLYFNELQNRTRDYTNHCVTAYNNGLEEIRGTSPASWLRYHQFRRETTLIALDLVAIFPYYNVREYPIGVNPQLTRDVYTDPIGVTFRREDWETGVECRPWVNTPYMSFSDLENAIIRPPHLFETLRNLTIHTGRYNLVGGARFIEGWVGHSVTNTRLGNSTVFTSNYGSLPPRFQVFNFTNFDVYQINTRADSTGTFRIPGFAVTRAQFIPGGTYSVAHRDPGACQQDYDSIEELPSLDPDEPINRSYSHRLSHVTLYKYTLSDTDYGVINYTDYGSMPAYVWTHRDVDLTNTITADRITQLPLVKASTLPAGTTVVKGPGFTGGDILRRTTNGTFGTLHVRVNSPLTQQYRLRVRFASTGNFSIRVLRGGTSIGDARFGSTMNRGQELTYESFVTREFTTTGPFNPPFTFTQTQEILTVNAEGVSTGGEYYIDSIEIVPVNPTREAEEDLEAAKKAVASLFTRTRDGLQVNVTDYQVDQAANLVSCLSDEQYGHDKKMLLEAVRAAKRLSRERNLLQDPDFNTINSTEENGWKASNGVTISEGGPFYKGRALQLASARENYPTYIYQKVNASELKPYTRYRLDGFVKSSQDLEIDLIHHHKVHLVKNVPDNLVSDTYSDGSCSGMNRCEEQQMVNAQLETEHHHPMDCCEAAQTHEFSSYINTGDLNSSVDQGIWVVLKVRTTDGYATLGNLELVEVGPLSGESLEREQRDNAKWSAELGRKRAETDRVYQDAKQSINHLFVDYQDQQLNPEIGMADIIDAQNLVASISDVYSDAVLQIPGINYEIYTELSNRLQQASYLYTSRNAVQNGDFNSGLDSWNATGGATVQQDGNTHFLVLSHWDAQVSQQFRVQPNCKYVLRVTAEKVGGGDGYVTIRDGAHHTEKLTFNACDYDINGTYVTDNTYLTKEVVFYSHTEHMWVEVSETEGAFHIDSIEFVETEK

SEQ ID NO: 7 - protein, 1127 aa, Bacillus thuringiensis
MSDGDYVDSYINPGLSIGRRDVTLTGVGIVALIVGTLGGPVGGIVTGLISSLLGLLWPSNDNDVWEAFMAQIEELIEQRIADQVVRNALDNLTGLRDYYNQYLLALEEWQERPNAVRSTLVFNRFETLHSHFVTSMPSFGSGPGSERYAVQLLTVYAQAANLHLLLLRDADIYGARWGLRESQIDLYFNELQNRTRDYTNHCVTAYNNGLEEIRGTSPASWLRYHQFRRETTLIALDLVAIFPYYNVREYPIGVNPQLTRDVYTDPIGVTFRREDWETGVECRPWVNTPYMSFSDLENAIIRPPHLFETLRNLTIHTGRYNLVGGARFIEGWVGHSVTNTRLGNSTVFTSNYGSLPPRFQVFNFTNFDVYQINTRADSTGTFRIPGFAVTRAQFIPGGTYSVAHRDPGACQQDYDSIEELPSLDPDEPINRSYSHRLSHVTLYKYTLSDTDYGVINYTDYGSMPAYVWTHRDVDLTNTITADRITQLPLVKASTLPAGTTVVKGPGFTGGDILRRTTNGTFGTLHVRVNSPLTQQYRLRVRFASTGNFSIRVLRGGTSIGDARFGSTMNRGQELTYESFVTREFTTTGPFNPPFTFTQTQEILTVNAEGVSTGGEYYIDSIEIVPVNPTREAEEDLEAAKKAVASLFTRTRDGLQVNVTDYQVDQAANLVSCLSDEQYGHDKKMLLEAVRAAKRLSRERNLLQDPDFNTINSTEENGWKASNGVTISEGGPFYKGRALQLASARENYPTYIYQKVNASELKPYTRYRLDGFVKSSQDLEIDLIHHHKVHLVKNVPDNLVSDTYSDGSCSGMNRCEEQQMVNAQLETEHHHPMDCCEAAQTHEFSSYINTGDLNSSVDQGIWVVLKVRTTDGYATLGNLELVEVGPLSGESLEREQRDNAKWSAELGRKRAETDRVYQDAKQSINHLFVDYQDQQLNPEIGMADIIDAQNLVASISDVYSDAVLQIPGINYEIYTELSNRLQQASYLYTSRNAVQNGDFNSGLDSWNATGGATVQQDGNTHFLVLSHWDAQVSQQFRVQPNCKYVLRVTAEKVGGGDGYVTIRDGAHHTEKLTFNACDYDINGTYVTDNTYLTKEVVFYSHTEHMWVEVSETEGAFHIDSIEFVETEK

SEQ ID NO: 8 - protein, 673 aa, Bacillus thuringiensis
MNRNNQGEYEIIDASTCGCSSDDVVQYPLARDPNAAFQNMNYKDYLKMSDGDYVDSYINPGLSIGRRDVTLTGVGIVALIVGTLGGPVGGIVTGLISSLLGLLWPSNDNDVWEAFMAQIEELIEQRIADQVVRNALDNLTGLRDYYNQYLLALEEWQERPNAVRSTLVFNRFETLHSHFVTSMPSFGSGPGSERYAVQLLTVYAQAANLHLLLLRDADIYGARWGLRESQIDLYFNELQNRTRDYTNHCVTAYNNGLEEIRGTSPASWLRYHQFRRETTLIALDLVAIFPYYNVREYPIGVNPQLTRDVYTDPIGVTFRREDWETGVECRPWVNTPYMSFSDLENAIIRPPHLFETLRNLTIHTGRYNLVGGARFIEGWVGHSVTNTRLGNSTVFTSNYGSLPPRFQVFNFTNFDVYQINTRADSTGTFRIPGFAVTRAQFIPGGTYSVAHRDPGACQQDYDSIEELPSLDPDEPINRSYSHRLSHVTLYKYTLSDTDYGVINYTDYGSMPAYVWTHRDVDLTNTITADRITQLPLVKASTLPAGTTVVKGPGFTGGDILRRTTNGTFGTLHVRVNSPLTQQYRLRVRFASTGNFSIRVLRGGTSIGDARFGSTMNRGQELTYESFVTREFTTTGPFNPPFTFTQTQEILTVNAEGVSTGGEYYIDSIEIVPV

SEQ ID NO: 9 - protein, 634 aa, Bacillus thuringiensis
MNYKDYLKMSDGDYVDSYINPGLSIGRRDVTLTGVGIVALIVGTLGGPVGGIVTGLISSLLGLLWPSNDNDVWEAFMAQIEELIEQRIADQVVRNALDNLTGLRDYYNQYLLALEEWQERPNAVRSTLVFNRFETLHSHFVTSMPSFGSGPGSERYAVQLLTVYAQAANLHLLLLRDADIYGARWGLRESQIDLYFNELQNRTRDYTNHCVTAYNNGLEEIRGTSPASWLRYHQFRRETTLIALDLVAIFPYYNVREYPIGVNPQLTRDVYTDPIGVTFRREDWETGVECRPWVNTPYMSFSDLENAIIRPPHLFETLRNLTIHTGRYNLVGGARFIEGWVGHSVTNTRLGNSTVFTSNYGSLPPRFQVFNFTNFDVYQINTRADSTGTFRIPGFAVTRAQFIPGGTYSVAHRDPGACQQDYDSIEELPSLDPDEPINRSYSHRLSHVTLYKYTLSDTDYGVINYTDYGSMPAYVWTHRDVDLTNTITADRITQLPLVKASTLPAGTTVVKGPGFTGGDILRRTTNGTFGTLHVRVNSPLTQQYRLRVRFASTGNFSIRVLRGGTSIGDARFGSTMNRGQELTYESFVTREFTTTGPFNPPFTFTQTQEILTVNAEGVSTGGEYYIDSIEIVPV

SEQ ID NO: 10 - protein, 626 aa, Bacillus thuringiensis
MSDGDYVDSYINPGLSIGRRDVTLTGVGIVALIVGTLGGPVGGIVTGLISSLLGLLWPSNDNDVWEAFMAQIEELIEQRIADQVVRNALDNLTGLRDYYNQYLLALEEWQERPNAVRSTLVFNRFETLHSHFVTSMPSFGSGPGSERYAVQLLTVYAQAANLHLLLLRDADIYGARWGLRESQIDLYFNELQNRTRDYTNHCVTAYNNGLEEIRGTSPASWLRYHQFRRETTLIALDLVAIFPYYNVREYPIGVNPQLTRDVYTDPIGVTFRREDWETGVECRPWVNTPYMSFSDLENAIIRPPHLFETLRNLTIHTGRYNLVGGARFIEGWVGHSVTNTRLGNSTVFTSNYGSLPPRFQVFNFTNFDVYQINTRADSTGTFRIPGFAVTRAQFIPGGTYSVAHRDPGACQQDYDSIEELPSLDPDEPINRSYSHRLSHVTLYKYTLSDTDYGVINYTDYGSMPAYVWTHRDVDLTNTITADRITQLPLVKASTLPAGTTVVKGPGFTGGDILRRTTNGTFGTLHVRVNSPLTQQYRLRVRFASTGNFSIRVLRGGTSIGDARFGSTMNRGQELTYESFVTREFTTTGPFNPPFTFTQTQEILTVNAEGVSTGGEYYIDSIEIVPV

SEQ ID NO: 11 - protein, 336 aa, Bacillus thuringiensis
MNKKVTKTVLSVVMGISVLASPLAVAAKTENNKEQQVITQFNQRENKFPDVGQGIQWLSQFYGKSLKNNGEGYSLGNDVMSYFLEVKNSYGQLAIEPQVISTTPLWAGQSDLENATDHEQTLNSTEFKKTYSNTTTTSTENGFMIGQETEGKVGIPFVAEGKVTIKTEYNFNHTNGYETSESVEYIAPSQSIKVPPHTIARVTALLDVKKIKGKMHLYSEIGLNKDYGYDMVPLVYKYGGPFKYVTLGTLYDEGYKQAQLDYSNMGNVIPEEIETVSKSNNPNHLLASGLGIFESEYGSVFNVKVEYINIKTKKIEKTENLTIEPTIVPVEKTNTK

SEQ ID NO: 12 - protein, 323 aa, Bacillus thuringiensis
MGISVLASPLAVAAKTENNKEQQVITQFNQRENKFPDVGQGIQWLSQFYGKSLKNNGEGYSLGNDVMSYFLEVKNSYGQLAIEPQVISTTPLWAGQSDLENATDHEQTLNSTEFKKTYSNTTTTSTENGFMIGQETEGKVGIPFVAEGKVTIKTEYNFNHTNGYETSESVEYIAPSQSIKVPPHTIARVTALLDVKKIKGKMHLYSEIGLNKDYGYDMVPLVYKYGGPFKYVTLGTLYDEGYKQAQLDYSNMGNVIPEEIETVSKSNNPNHLLASGLGIFESEYGSVFNVKVEYINIKTKKIEKTENLTIEPTIVPVEKTNTK

SEQ ID NO: 13 - protein, 310 aa, Bacillus thuringiensis
MKTENNKEQQVITQFNQRENKFPDVGQGIQWLSQFYGKSLKNNGEGYSLGNDVMSYFLEVKNSYGQLAIEPQVISTTPLWAGQSDLENATDHEQTLNSTEFKKTYSNTTTTSTENGFMIGQETEGKVGIPFVAEGKVTIKTEYNFNHTNGYETSESVEYIAPSQSIKVPPHTIARVTALLDVKKIKGKMHLYSEIGLNKDYGYDMVPLVYKYGGPFKYVTLGTLYDEGYKQAQLDYSNMGNVIPEEIETVSKSNNPNHLLASGLGIFESEYGSVFNVKVEYINIKTKKIEKTENLTIEPTIVPVEKTNTK

SEQ ID NO: 14 - protein, 257 aa, Bacillus thuringiensis
MSYFLEVKNSYGQLAIEPQVISTTPLWAGQSDLENATDHEQTLNSTEFKKTYSNTTTTSTENGFMIGQETEGKVGIPFVAEGKVTIKTEYNFNHTNGYETSESVEYIAPSQSIKVPPHTIARVTALLDVKKIKGKMHLYSEIGLNKDYGYDMVPLVYKYGGPFKYVTLGTLYDEGYKQAQLDYSNMGNVIPEEIETVSKSNNPNHLLASGLGIFESEYGSVFNVKVEYINIKTKKIEKTENLTIEPTIVPVEKTNTK

SEQ ID NO: 15 - protein, 341 aa, Bacillus thuringiensis
MREKDLNKKVTKAVLSMIVGISVLASPLAVAAKTENNKEQQVITHFNQRENKFPDVGQGIQWLSQFYGKSLKNNGEGYSLGQDVMRYFLEVKNSYGQLAMEPQVISTTPLWAGQSDLENATDHEQTLNSTEFKKTYSNTTTTSTENGFMIGQETEGKVGIPFVAEGKVTIKTEYNFNHTNGYETSESVEYIAPSQSIKVPPHTIARVTALLDVKKIKGKMHLYSEIGLNKDYGYDMVPLVYKYGGPFKYVTLGTLYDEGYKQAQLDYFNMGNVIPEEIETVSKSNNPNHLLASGVGIFESEYGSVFNVKVEYININTKKIEKTENLTIEPTIVPVKQTNTK

SEQ ID NO: 16 - protein, 325 aa, Bacillus thuringiensis
MIVGISVLASPLAVAAKTENNKEQQVITHFNQRENKFPDVGQGIQWLSQFYGKSLKNNGEGYSLGQDVMRYFLEVKNSYGQLAMEPQVISTTPLWAGQSDLENATDHEQTLNSTEFKKTYSNTTTTSTENGFMIGQETEGKVGIPFVAEGKVTIKTEYNFNHTNGYETSESVEYIAPSQSIKVPPHTIARVTALLDVKKIKGKMHLYSEIGLNKDYGYDMVPLVYKYGGPFKYVTLGTLYDEGYKQAQLDYFNMGNVIPEEIETVSKSNNPNHLLASGVGIFESEYGSVFNVKVEYININTKKIEKTENLTIEPTIVPVKQTNTK

SEQ ID NO: 17 - protein, 315 aa, Bacillus thuringiensis
MLAVAAKTENNKEQQVITHFNQRENKFPDVGQGIQWLSQFYGKSLKNNGEGYSLGQDVMRYFLEVKNSYGQLAMEPQVISTTPLWAGQSDLENATDHEQTLNSTEFKKTYSNTTTTSTENGFMIGQETEGKVGIPFVAEGKVTIKTEYNFNHTNGYETSESVEYIAPSQSIKVPPHTIARVTALLDVKKIKGKMHLYSEIGLNKDYGYDMVPLVYKYGGPFKYVTLGTLYDEGYKQAQLDYFNMGNVIPEEIETVSKSNNPNHLLASGVGIFESEYGSVFNVKVEYININTKKIEKTENLTIEPTIVPVKQTNTK

SEQ ID NO: 18 - protein, 257 aa, Bacillus thuringiensis
MRYFLEVKNSYGQLAMEPQVISTTPLWAGQSDLENATDHEQTLNSTEFKKTYSNTTTTSTENGFMIGQETEGKVGIPFVAEGKVTIKTEYNFNHTNGYETSESVEYIAPSQSIKVPPHTIARVTALLDVKKIKGKMHLYSEIGLNKDYGYDMVPLVYKYGGPFKYVTLGTLYDEGYKQAQLDYFNMGNVIPEEIETVSKSNNPNHLLASGVGIFESEYGSVFNVKVEYININTKKIEKTENLTIEPTIVPVKQTNTK

SEQ ID NO: 19 - protein, 242 aa, Bacillus thuringiensis
MEPQVISTTPLWAGQSDLENATDHEQTLNSTEFKKTYSNTTTTSTENGFMIGQETEGKVGIPFVAEGKVTIKTEYNFNHTNGYETSESVEYIAPSQSIKVPPHTIARVTALLDVKKIKGKMHLYSEIGLNKDYGYDMVPLVYKYGGPFKYVTLGTLYDEGYKQAQLDYFNMGNVIPEEIETVSKSNNPNHLLASGVGIFESEYGSVFNVKVEYININTKKIEKTENLTIEPTIVPVKQTNTK

SEQ ID NO: 20 - protein, 343 aa, Bacillus thuringiensis
MREKDMDKKITKAALSMIMGISVLSSPLAVAAKTENNKEQHVITQFNQRENKFPDVGQGIQWLSQFYGKSLKNNGEGYSLGQDVMSYFLEVKNSYGQLAMEPQVISTTPLWAGQSDLENATDHEQTLNSTEFKKTYSNTTTTSTENGFMIGQETEGKVGIPFVAEGKVTIKTEYNFNHTNGYETSESVEYIAPSQSIKVPPHTIARVTALLDVKKIKGKMHLYSEIGLNKDYGYDMVPLVYKYGGPFKYVTLGTLYDEGYKQAQLDYFNMGNVIPEEIETVSKSNNPNHLLASGVGIFESEYGSVFNVKVEYININTKKIEKTENLTIEPTIVPVKQTNTNTK

SEQ ID NO: 21 - protein, 338 aa, Bacillus thuringiensis
MDKKITKAALSMIMGISVLSSPLAVAAKTENNKEQHVITQFNQRENKFPDVGQGIQWLSQFYGKSLKNNGEGYSLGQDVMSYFLEVKNSYGQLAMEPQVISTTPLWAGQSDLENATDHEQTLNSTEFKKTYSNTTTTSTENGFMIGQETEGKVGIPFVAEGKVTIKTEYNFNHTNGYETSESVEYIAPSQSIKVPPHTIARVTALLDVKKIKGKMHLYSEIGLNKDYGYDMVPLVYKYGGPFKYVTLGTLYDEGYKQAQLDYFNMGNVIPEEIETVSKSNNPNHLLASGVGIFESEYGSVFNVKVEYININTKKIEKTENLTIEPTIVPVKQTNTNTK

SEQ ID NO: 22 - protein, 327 aa, Bacillus thuringiensis
MIMGISVLSSPLAVAAKTENNKEQHVITQFNQRENKFPDVGQGIQWLSQFYGKSLKNNGEGYSLGQDVMSYFLEVKNSYGQLAMEPQVISTTPLWAGQSDLENATDHEQTLNSTEFKKTYSNTTTTSTENGFMIGQETEGKVGIPFVAEGKVTIKTEYNFNHTNGYETSESVEYIAPSQSIKVPPHTIARVTALLDVKKIKGKMHLYSEIGLNKDYGYDMVPLVYKYGGPFKYVTLGTLYDEGYKQAQLDYFNMGNVIPEEIETVSKSNNPNHLLASGVGIFESEYGSVFNVKVEYININTKKIEKTENLTIEPTIVPVKQTNTNTK

SEQ ID NO: 23 - protein, 325 aa, Bacillus thuringiensis
MGISVLSSPLAVAAKTENNKEQHVITQFNQRENKFPDVGQGIQWLSQFYGKSLKNNGEGYSLGQDVMSYFLEVKNSYGQLAMEPQVISTTPLWAGQSDLENATDHEQTLNSTEFKKTYSNTTTTSTENGFMIGQETEGKVGIPFVAEGKVTIKTEYNFNHTNGYETSESVEYIAPSQSIKVPPHTIARVTALLDVKKIKGKMHLYSEIGLNKDYGYDMVPLVYKYGGPFKYVTLGTLYDEGYKQAQLDYFNMGNVIPEEIETVSKSNNPNHLLASGVGIFESEYGSVFNVKVEYININTKKIEKTENLTIEPTIVPVKQTNTNTK

SEQ ID NO: 24 - protein, 259 aa, Bacillus thuringiensis
MSYFLEVKNSYGQLAMEPQVISTTPLWAGQSDLENATDHEQTLNSTEFKKTYSNTTTTSTENGFMIGQETEGKVGIPFVAEGKVTIKTEYNFNHTNGYETSESVEYIAPSQSIKVPPHTIARVTALLDVKKIKGKMHLYSEIGLNKDYGYDMVPLVYKYGGPFKYVTLGTLYDEGYKQAQLDYFNMGNVIPEEIETVSKSNNPNHLLASGVGIFESEYGSVFNVKVEYININTKKIEKTENLTIEPTIVPVKQTNTNTK

SEQ ID NO: 25 - protein, 244 aa, Bacillus thuringiensis
MEPQVISTTPLWAGQSDLENATDHEQTLNSTEFKKTYSNTTTTSTENGFMIGQETEGKVGIPFVAEGKVTIKTEYNFNHTNGYETSESVEYIAPSQSIKVPPHTIARVTALLDVKKIKGKMHLYSEIGLNKDYGYDMVPLVYKYGGPFKYVTLGTLYDEGYKQAQLDYFNMGNVIPEEIETVSKSNNPNHLLASGVGIFESEYGSVFNVKVEYININTKKIEKTENLTIEPTIVPVKQTNTNTK

SEQ ID NO: 26 - protein, 312 aa, Bacillus thuringiensis
MKTENNKEQHVITQFNQRENKFPDVGQGIQWLSQFYGKSLKNNGEGYSLGQDVMSYFLEVKNSYGQLAMEPQVISTTPLWAGQSDLENATDHEQTLNSTEFKKTYSNTTTTSTENGFMIGQETEGKVGIPFVAEGKVTIKTEYNFNHTNGYETSESVEYIAPSQSIKVPPHTIARVTALLDVKKIKGKMHLYSEIGLNKDYGYDMVPLVYKYGGPFKYVTLGTLYDEGYKQAQLDYFNMGNVIPEEIETVSKSNNPNHLLASGVGIFESEYGSVFNVKVEYININTKKIEKTENLTIEPTIVPVKQTNTNTK

SEQ ID NO: 27 - protein, 4 aa, Artificial Sequence
  Endoplasmic reticulum targeting peptide
KDEL